European Patent Application EP 4 190 355 A1, published June 7, 2023. Title: FORMULATIONS OF HUMAN ANTI-RANKL ANTIBODIES, AND METHODS OF USING THE SAME. Applicant: Amgen Inc. The sequence listing filed with the application follows.

SEQUENCE LISTING (27 sequences)

SEQ ID NO: 1 - protein, 108 aa, Homo sapiens
  source 1..108: note = denosumab variable light chain
EIVLTQSPGTLSLSPGERATLSCRASQSVRGRYLAWYQQKPGQAPRLLIYGASSRATGIPDRFSGSGSGTDFTLTISRLEPEDFAVFYCQQYGSSPRTFGQGTKVEIK

SEQ ID NO: 2 - protein, 122 aa, Homo sapiens
  source 1..122: note = denosumab variable heavy chain
EVQLLESGGGLVQPGGSLRLSCAASGFTFSSYAMSWVRQAPGKGLEWVSGITGSGGSTYYADSVKGRFTISRDNSKNTLYLQMNSLRAEDTAVYYCAKDPGTTVIMSWFDPWGQGTLVTVSS

SEQ ID NO: 3 - protein, 235 aa, Homo sapiens
  source 1..235: note = denosumab full length light chain
METPAQLLFLLLLWLPDTTGEIVLTQSPGTLSLSPGERATLSCRASQSVRGRYLAWYQQKPGQAPRLLIYGASSRATGIPDRFSGSGSGTDFTLTISRLEPEDFAVFYCQQYGSSPRTFGQGTKVEIKRTVAAPSVFIFPPSDEQLKSGTASVVCLLNNFYPREAKVQWKVDNALQSGNSQESVTEQDSKDSTYSLSSTLTLSKADYEKHKVYACEVTHQGLSSPVTKSFNRGEC

SEQ ID NO: 4 - protein, 467 aa, Homo sapiens
  source 1..467: note = denosumab full length heavy chain
MEFGLSWLFLVAILKGVQCEVQLLESGGGLVQPGGSLRLSCAASGFTFSSYAMSWVRQAPGKGLEWVSGITGSGGSTYYADSVKGRFTISRDNSKNTLYLQMNSLRAEDTAVYYCAKDPGTTVIMSWFDPWGQGTLVTVSSASTKGPSVFPLAPCSRSTSESTAALGCLVKDYFPEPVTVSWNSGALTSGVHTFPAVLQSSGLYSLSSVVTVPSSNFGTQTYTCNVDHKPSNTKVDKTVERKCCVECPPCPAPPVAGPSVFLFPPKPKDTLMISRTPEVTCVVVDVSHEDPEVQFNWYVDGVEVHNAKTKPREEQFNSTFRVVSVLTVVHQDWLNGKEYKCKVSNKGLPAPIEKTISKTKGQPREPQVYTLPPSREEMTKNQVSLTCLVKGFYPSDIAVEWESNGQPENNYKTTPPMLDSDGSFFLYSKLTVDKSRWQQGNVFSCSVMHEALHNHYTQKSLSLSPGK

SEQ ID NO: 5 - protein, 12 aa, Homo sapiens
  source 1..12: note = Light Chain CDR 1
RASQSVRGRYLA

SEQ ID NO: 6 - protein, 7 aa, Homo sapiens
  source 1..7: note = Light Chain CDR 2
GASSRAT

SEQ ID NO: 7 - protein, 9 aa, Homo sapiens
  source 1..9: note = Light Chain CDR 3
QQYGSSPRT

SEQ ID NO: 8 - protein, 5 aa, Homo sapiens
  source 1..5: note = Heavy Chain CDR 1
SYAMS

SEQ ID NO: 9 - protein, 17 aa, Homo sapiens
  source 1..17: note = Heavy Chain CDR 2
GITGSGGSTYYADSVKG

SEQ ID NO: 10 - protein, 13 aa, Homo sapiens
  source 1..13: note = Heavy Chain CDR 3
DPGTTVIMSWFDP

SEQ ID NO: 11 - DNA, 2141 bp, Homo sapiens
  source 1..2141: mol_type = genomic DNA
ggccaaagccgggctccaagtcggcgccccacgtcgaggctccgccgcagcctccggagttggccgcagacaagaaggggagggagcgggagagggaggagagctccgaagcgagagggccgagcgccatgcgccgcgccagcagagactacaccaagtacctgcgtggctcggaggagatgggcggcggccccggagccccgcacgagggccccctgcacgccccgccgccgcctgcgccgcaccagccccccgccgcctcccgctccatgttcgtggccctcctggggctggggctgggccaggttgtctgcagcgtcgccctgttcttctatttcagagcgcagatggatcctaatagaatatcagaagatggcactcactgcatttatagaattttgagactccatgaaaatgcagattttcaagacacaactctggagagtcaagatacaaaattaatacctgattcatgtaggagaattaaacaggcctttcaaggagctgtgcaaaaggaattacaacatatcgttggatcacagcacatcagagcagagaaagcgatggtggatggctcatggttagatctggccaagaggagcaagcttgaagctcagccttttgctcatctcactattaatgccaccgacatcccatctggttcccataaagtgagtctgtcctcttggtaccatgatcggggttgggccaagatctccaacatgacttttagcaatggaaaactaatagttaatcaggatggcttttattacctgtatgccaacatttgctttcgacatcatgaaacttcaggagacctagctacagagtatcttcaactaatggtgtacgtcactaaaaccagcatcaaaatcccaagttctcataccctgatgaaaggaggaagcaccaagtattggtcagggaattctgaattccatttttattccataaacgttggtggattttttaagttacggtctggagaggaaatcagcatcgaggtctccaacccctccttactggatccggatcaggatgcaacatactttggggcttttaaagttcgagatatagattgagccccagtttttggagtgttatgtatttcctggatgtttggaaacattttttaaaacaagccaagaaagatgtatataggtgtgtgagactactaagaggcatggccccaacggtacacgactcagtatccatgctcttgaccttgtagagaacacgcgtatttacctgccagtgggagatgttagactcatggtgtgttacacaatggtttttaaattttgtaatgaattcctagaattaaaccagattggagcaattacgggttgaccttatgagaaactgcatgtgggctatgggaggggttggtccctggtcatgtgccccttcgcagctgaagtggagagggtgtcatctagcgcaattgaaggatcatctgaaggggcaaattcttttgaattgttacatcatgctggaacctgcaaaaaatactttttctaatgaggagagaaaatatatgtatttttatataatatctaaagttatatttcagatgtaatgttttctttgcaaagtattgtaaattatatttgtgctataacagacatatttaactggtgcactttgtaaattccctggggaaaacttgcagctaaggaggggaaaaaaatgttgtttcctaatatcaaatgcagtatatttcttcgttctttttaagttaatagattttttcagacttgtcaagcctgtgcaaaaaaattaaaatggatgccttgaataataagcaggatgttggccaccaggtgcctttcaaatttagaaactaattgactttagaaagctgacattgccaaaaaggatacataatgggccactgaaatttgtcaagagtagttatataattgttgaacaggtgtttttccacaagtgccgcaaattgtacctttttttttttttcaaaatagaaaagttattagtggtttatcagcaaaaaagtccaattttaatttagtaaatgttattttatactgtacaataaaaacattgcctttgaatgttaattttttggtacaaaaataaatttatatgaaaaaaaaaaaaaaaaaaaaaaaaaaaaaaaa

SEQ ID NO: 12 - protein, 317 aa, Homo sapiens
MRRASRDYTKYLRGSEEMGGGPGAPHEGPLHAPPPPAPHQPPAASRSMFVALLGLGLGQVVCSVALFFYFRAQMDPNRISEDGTHCIYRILRLHENADFQDTTLESQDTKLIPDSCRRIKQAFQGAVQKELQHIVGSQHIRAEKAMVDGSWLDLAKRSKLEAQPFAHLTINATDIPSGSHKVSLSSWYHDRGWAKISNMTFSNGKLIVNQDGFYYLYANICFRHHETSGDLATEYLQLMVYVTKTSIKIPSSHTLMKGGSTKYWSGNSEFHFYSINVGGFFKLRSGEEISIEVSNPSLLDPDQDATYFGAFKVRDID

SEQ ID NO: 13 - protein, 215 aa, synthetic construct
  source 1..215: note = Synthetic Polypeptide
EIVLTQSPGTLSLSPGERATLSCRASQSVRGRYLAWYQQKPGQAPRLLIYGASSRATGIPDRFSGSGSGTDFTLTISRLEPEDFAVFYCQQYGSSPRTFGQGTKVEIKRTVAAPSVFIFPPSDEQLKSGTASVVCLLNNFYPREAKVQWKVDNALQSGNSQESVTEQDSKDSTYSLSSTLTLSKADYEKHKVYACEVTHQGLSSPVTKSFNRGEC

SEQ ID NO: 14 - protein, 448 aa, synthetic construct
  source 1..448: note = Synthetic Polypeptide
EVQLLESGGGLVQPGGSLRLSCAASGFTFSSYAMSWVRQAPGKGLEWVSGITGSGGSTYYADSVKGRFTISRDNSKNTLYLQMNSLRAEDTAVYYCAKDPGTTVIMSWFDPWGQGTLVTVSSASTKGPSVFPLAPCSRSTSESTAALGCLVKDYFPEPVTVSWNSGALTSGVHTFPAVLQSSGLYSLSSVVTVPSSNFGTQTYTCNVDHKPSNTKVDKTVERKCCVECPPCPAPPVAGPSVFLFPPKPKDTLMISRTPEVTCVVVDVSHEDPEVQFNWYVDGVEVHNAKTKPREEQFNSTFRVVSVLTVVHQDWLNGKEYKCKVSNKGLPAPIEKTISKTKGQPREPQVYTLPPSREEMTKNQVSLTCLVKGFYPSDIAVEWESNGQPENNYKTTPPMLDSDGSFFLYSKLTVDKSRWQQGNVFSCSVMHEALHNHYTQKSLSLSPGK

SEQ ID NO: 15 - protein, 330 aa, synthetic construct
  VARIANT 14: note = Cys or Ser
  VARIANT 100: note = Ser, Arg, or Pro
  VARIANT 117: note = Phe, Val, or Leu
  source 1..330: note = Synthetic Polypeptide
  VARIANT 16: note = Arg or Lys
  VARIANT 20: note = Glu or Gly
  VARIANT 21: note = Ser or Gly
  VARIANT 75: note = Ser or Asn
  VARIANT 76: note = Leu or Phe
  VARIANT 79: note = Lys or Gln
  VARIANT 82: note = Thr or Ile
  VARIANT 97: note = Arg, Thr, or Lys
  VARIANT 102: note = Tyr, Cys, or Ser
  VARIANT 103: note = Gly or Cys
  VARIANT 104: note = absent or Asp
  VARIANT 105: note = absent or Lys
  VARIANT 106: note = absent or Thr
  VARIANT 107: note = Pro, Val or His
  VARIANT 108: note = Pro, Glu, or Thr
  VARIANT 111: note = Ser or Pro
  VARIANT 116: note = Glu or Pro
  VARIANT 118: note = Leu or Ala
  VARIANT 120: note = absent or Gly
  VARIANT 151: note = Gln or His
  VARIANT 157: note = Gln or Lys
  VARIANT 179: note = Phe or Tyr
  VARIANT 183: note = Tyr or Phe
  VARIANT 192: note = Leu or Val
  VARIANT 210: note = Gly or Ala
  VARIANT 213: note = Ser or Ala
  VARIANT 214: note = Ser or Pro
  VARIANT 222: note = Ala or Thr
  VARIANT 238: note = Gln or Arg
  VARIANT 239: note = Glu or Asp
  VARIANT 241: note = Met or Leu
  VARIANT 280: note = Val or Met
  VARIANT 292: note = Arg or Lys
  VARIANT 328: note = Leu or Pro
ASTKGPSVFPLAPXSXSTSXXTAALGCLVKDYFPEPVTVSWNSGALTSGVHTFPAVLQSSGLYSLSSVVTVPSSXXGTXTYXCNVBHKPSNTKVDKXVEXKXXXXXXXCPXCPAPXXXGXPSVFLFPPKPKDTLMISRTPEVTCVVVDVSXEDPEVXFNWYVDGVEVHNAKTKPREEQXNSTXRVVSVLTVXHQDWLNGKEYKCKVSNKXLPXXIEKTISKXKGQPREPQVYTLPPSXXEXTKNQVSLTCLVKGFYPSDIAVEWESNGQPENNYKTTPPXLDSDGSFFLYSXLTVDKSRWQZGNVFSCSVMHEALHNHYTQKSLSLSXGK

SEQ ID NO: 16 - protein, 326 aa, synthetic construct
  source 1..326: note = IgG2 Constant HC; note = Synthetic Polypeptide
ASTKGPSVFPLAPCSRSTSESTAALGCLVKDYFPEPVTVSWNSGALTSGVHTFPAVLQSSGLYSLSSVVTVPSSNFGTQTYTCNVDHKPSNTKVDKTVERKCCVECPPCPAPPVAGPSVFLFPPKPKDTLMISRTPEVTCVVVDVSHEDPEVQFNWYVDGVEVHNAKTKPREEQFNSTFRVVSVLTVVHQDWLNGKEYKCKVSNKGLPAPIEKTISKTKGQPREPQVYTLPPSREEMTKNQVSLTCLVKGFYPSDIAVEWESNGQPENNYKTTPPMLDSDGSFFLYSKLTVDKSRWQQGNVFSCSVMHEALHNHYTQKSLSLSPGK

SEQ ID NO: 17 - protein, 330 aa, synthetic construct [sequence omitted]

SEQ ID NO: 18 - protein, 327 aa, synthetic construct
  source 1..327: note = IgG4 constant HC; note = Synthetic Polypeptide
ASTKGPSVFPLAPCSRSTSESTAALGCLVKDYFPEPVTVSWNSGALTSGVHTFPAVLQSSGLYSLSSVVTVPSSSLGTKTYTCNVDHKPSNTKVDKRVESKYGPPCPSCPAPEFLGGPSVFLFPPKPKDTLMISRTPEVTCVVVDVSQEDPEVQFNWYVDGVEVHNAKTKPREEQFNSTYRVVSVLTVLHQDWLNGKEYKCKVSNKGLPSSIEKTISKAKGQPREPQVYTLPPSQEEMTKNQVSLTCLVKGFYPSDIAVEWESNGQPENNYKTTPPVLDSDGSFFLYSRLTVDKSRWQEGNVFSCSVMHEALHNHYTQKSLSLSLGK

SEQ ID NO: 19 - DNA, 324 bp, synthetic construct
  source 1..324: mol_type = other DNA; note = variable LC; note = Synthetic Polynucleotide
gaaattgtgttgacgcagtctccaggcaccctgtctttgtctccaggggaaagagccaccctctcctgtagggccagtcagagtgttcgcggcaggtacttagcctggtaccagcagaaacctggccaggctcccaggctcctcatctatggtgcatccagcagggccactggcatcccagacaggttcagtggcagtgggtctgggacagacttcactctcaccatcagcagactggagcctgaagattttgcagtgttttactgtcagcagtatggtagttcacctcggacgttcggccaagggaccaaggtggaaatcaaa

SEQ ID NO: 20 - DNA, 366 bp, synthetic construct
  source 1..366: mol_type = other DNA; note = variable HC; note = Synthetic Polynucleotide
gaggtgcagctgttggagtctgggggaggcttggtacagcctggggggtccctgagactctcctgtgcagcctctggattcacctttagcagctatgccatgagctgggtccgccaggctccagggaaggggctggagtgggtctcaggtattactgggagtggtggtagtacatactacgcagactccgtgaagggccggttcaccatctccagagacaattccaagaacacgctgtatctgcaaatgaacagcctgagagccgaggacacggccgtatattactgtgcgaaagatccagggactacggtgattatgagttggttcgacccctggggccagggaaccctggtcaccgtctcctca

SEQ ID NO: 21 - DNA, 705 bp, synthetic construct
  source 1..705: mol_type = other DNA; note = full length LC; note = Synthetic Polynucleotide
atggaaaccccagcgcagcttctcttcctcctgctactctggctcccagataccaccggagaaattgtgttgacgcagtctccaggcaccctgtctttgtctccaggggaaagagccaccctctcctgtagggccagtcagagtgttcgcggcaggtacttagcctggtaccagcagaaacctggccaggctcccaggctcctcatctatggtgcatccagcagggccactggcatcccagacaggttcagtggcagtgggtctgggacagacttcactctcaccatcagcagactggagcctgaagattttgcagtgttttactgtcagcagtatggtagttcacctcggacgttcggccaagggaccaaggtggaaatcaaacgaactgtggctgcaccatctgtcttcatcttcccgccatctgatgagcagttgaaatctggaactgcctctgttgtgtgcctgctgaataacttctatcccagagaggccaaagtacagtggaaggtggataacgccctccaatcgggtaactcccaggagagtgtcacagagcaggacagcaaggacagcacctacagcctcagcagcaccctgacgctgagcaaagcagactacgagaaacacaaagtctacgcctgcgaagtcacccatcagggcctgagctcgcccgtcacaaagagcttcaacaggggagagtgt

SEQ ID NO: 22 - DNA, 1401 bp, synthetic construct
  source 1..1401: mol_type = other DNA; note = full length HC; note = Synthetic Polynucleotide
atggagtttgggctgagctggctttttcttgtggctattttaaaaggtgtccagtgtgaggtgcagctgttggagtctgggggaggcttggtacagcctggggggtccctgagactctcctgtgcagcctctggattcacctttagcagctatgccatgagctgggtccgccaggctccagggaaggggctggagtgggtctcaggtattactgggagtggtggtagtacatactacgcagactccgtgaagggccggttcaccatctccagagacaattccaagaacacgctgtatctgcaaatgaacagcctgagagccgaggacacggccgtatattactgtgcgaaagatccagggactacggtgattatgagttggttcgacccctggggccagggaaccctggtcaccgtctcctcagcctccaccaagggcccatcggtcttccccctggcgccctgctccaggagcacctccgagagcacagcggccctgggctgcctggtcaaggactacttccccgaaccggtgacggtgtcgtggaactcaggcgctctgaccagcggcgtgcacaccttcccagctgtcctacagtcctcaggactctactccctcagcagcgtggtgaccgtgccctccagcaacttcggcacccagacctacacctgcaacgtagatcacaagcccagcaacaccaaggtggacaagacagttgagcgcaaatgttgtgtcgagtgcccaccgtgcccagcaccacctgtggcaggaccgtcagtcttcctcttccccccaaaacccaaggacaccctcatgatctcccggacccctgaggtcacgtgcgtggtggtggacgtgagccacgaagaccccgaggtccagttcaactggtacgtggacggcgtggaggtgcataatgccaagacaaagccacgggaggagcagttcaacagcacgttccgtgtggtcagcgtcctcaccgttgtgcaccaggactggctgaacggcaaggagtacaagtgcaaggtctccaacaaaggcctcccagcccccatcgagaaaaccatctccaaaaccaaagggcagccccgagaaccacaggtgtacaccctgcccccatcccgggaggagatgaccaagaaccaggtcagcctgacctgcctggtcaaaggcttctaccccagcgacatcgccgtggagtgggagagcaatgggcagccggagaacaactacaagaccacacctcccatgctggactccgacggctccttcttcctctacagcaagctcaccgtggacaagagcaggtggcagcaggggaacgtcttctcatgctccgtgatgcatgaggctctgcacaaccactacacgcagaagagcctctccctgtctccgggtaaa

SEQ ID NO: 23 - DNA, 645 bp, synthetic construct
  source 1..645: mol_type = other DNA; note = mature LC; note = Synthetic Polynucleotide
gaaattgtgttgacgcagtctccaggcaccctgtctttgtctccaggggaaagagccaccctctcctgtagggccagtcagagtgttcgcggcaggtacttagcctggtaccagcagaaacctggccaggctcccaggctcctcatctatggtgcatccagcagggccactggcatcccagacaggttcagtggcagtgggtctgggacagacttcactctcaccatcagcagactggagcctgaagattttgcagtgttttactgtcagcagtatggtagttcacctcggacgttcggccaagggaccaaggtggaaatcaaacgaactgtggctgcaccatctgtcttcatcttcccgccatctgatgagcagttgaaatctggaactgcctctgttgtgtgcctgctgaataacttctatcccagagaggccaaagtacagtggaaggtggataacgccctccaatcgggtaactcccaggagagtgtcacagagcaggacagcaaggacagcacctacagcctcagcagcaccctgacgctgagcaaagcagactacgagaaacacaaagtctacgcctgcgaagtcacccatcagggcctgagctcgcccgtcacaaagagcttcaacaggggagagtgt

SEQ ID NO: 24 - DNA, 1344 bp, synthetic construct
  source 1..1344: mol_type = other DNA; note = mature HC; note = Synthetic Polynucleotide
gaggtgcagctgttggagtctgggggaggcttggtacagcctggggggtccctgagactctcctgtgcagcctctggattcacctttagcagctatgccatgagctgggtccgccaggctccagggaaggggctggagtgggtctcaggtattactgggagtggtggtagtacatactacgcagactccgtgaagggccggttcaccatctccagagacaattccaagaacacgctgtatctgcaaatgaacagcctgagagccgaggacacggccgtatattactgtgcgaaagatccagggactacggtgattatgagttggttcgacccctggggccagggaaccctggtcaccgtctcctcagcctccaccaagggcccatcggtcttccccctggcgccctgctccaggagcacctccgagagcacagcggccctgggctgcctggtcaaggactacttccccgaaccggtgacggtgtcgtggaactcaggcgctctgaccagcggcgtgcacaccttcccagctgtcctacagtcctcaggactctactccctcagcagcgtggtgaccgtgccctccagcaacttcggcacccagacctacacctgcaacgtagatcacaagcccagcaacaccaaggtggacaagacagttgagcgcaaatgttgtgtcgagtgcccaccgtgcccagcaccacctgtggcaggaccgtcagtcttcctcttccccccaaaacccaaggacaccctcatgatctcccggacccctgaggtcacgtgcgtggtggtggacgtgagccacgaagaccccgaggtccagttcaactggtacgtggacggcgtggaggtgcataatgccaagacaaagccacgggaggagcagttcaacagcacgttccgtgtggtcagcgtcctcaccgttgtgcaccaggactggctgaacggcaaggagtacaagtgcaaggtctccaacaaaggcctcccagcccccatcgagaaaaccatctccaaaaccaaagggcagccccgagaaccacaggtgtacaccctgcccccatcccgggaggagatgaccaagaaccaggtcagcctgacctgcctggtcaaaggcttctaccccagcgacatcgccgtggagtgggagagcaatgggcagccggagaacaactacaagaccacacctcccatgctggactccgacggctccttcttcctctacagcaagctcaccgtggacaagagcaggtggcagcaggggaacgtcttctcatgctccgtgatgcatgaggctctgcacaaccactacacgcagaagagcctctccctgtctccgggtaaa

SEQ ID NO: 25 - protein, 20 aa, synthetic construct
  source 1..20: note = signal peptide of full length LC of SEQ 3; note = Synthetic Polypeptide
METPAQLLFLLLLWLPDTTG

SEQ ID NO: 26 - protein, 19 aa, synthetic construct
  source 1..19: note = signal peptide of full length HC of SEQ 4; note = Synthetic Polypeptide
MEFGLSWLFLVAILKGVQC

SEQ ID NO: 27 - protein, 10 aa, synthetic construct
  source 1..10: note = Synthetic Polypeptide
GFTFSSYAMS